European Patent Specification EP 3 782 625 B1, published October 23, 2024. Title: An agent for improving cytokine release syndrome, etc. Applicant: TORII PHARMACEUTICAL CO., LTD. The sequence listing filed with the application follows.

SEQUENCE LISTING (6 sequences)

SEQ ID NO: 1 - DNA, 35 bp, Artificial
  Synthetic DNA
cgctaccgtcgtcgaattcgccgccaccatgcttc

SEQ ID NO: 2 - DNA, 34 bp, Artificial
  Synthetic DNA
gaagttcgtgctccgggatcccgcgagggggcag

SEQ ID NO: 3 - DNA, 35 bp, Artificial
  Synthetic DNA
ccggttcgaattcgccatatgccacctcccgcctc

SEQ ID NO: 4 - DNA, 37 bp, Artificial
  Synthetic DNA
cgatgttaactctagatcacctgggtgctccaggtgc

SEQ ID NO: 5 - DNA, 26 bp, Artificial
  Synthetic DNA
gaattcgccaccatggaagatgccaa

SEQ ID NO: 6 - DNA, 24 bp, Artificial
  Synthetic DNA
ggatcccacggcgatcttgccgcc